European Patent Application EP 4 814 013 A1, published September 30, 2026. Title: 一种抗CD16a的单域抗体及其用途. Applicant: 南京融捷康生物科技有限公司. The sequence listing filed with the application follows.

SEQUENCE LISTING (70 sequences)

SEQ ID NO: 1 - protein, 126 aa, synthetic construct
QVQLVESGGGLVQAGGSLRLSCAASGGTFRIYAMGWFRQAPGKEREFVGSISMMRGITDYAESVKGRFTISRDNAKFTMYLQMNSLKSEDTAVYYCAKAVDKSPYGGWGWGPYDDWGQGTQVTVSS

SEQ ID NO: 2 - protein, 127 aa, synthetic construct
QVQLVESGGGLVQAGDSLRLSCAASGGTFRIYAMGWFRQAPGKEREFVGSISMMRGITDYAESVKGRFTISRDNAKFTMYLQMNTLKPEDTAVYYCAIRERPPPMGWGLAGISYDYWGQGTQVTVSS

SEQ ID NO: 3 - protein, 127 aa, synthetic construct
QVQLVESGGGLVQPGGSLRLSCAASGRTFRIYAMGWFRQAPGKEREFVGSIRLMRGITDYADSVKGRFTISRDNAKFTMYLQMNTLKPEDTAVYYCAAVGSGGDFYTPSTSGEYRYWGQGTQVTVSS

SEQ ID NO: 4 - protein, 126 aa, synthetic construct
QVQLVESGGGLVQPGGSLRLSCEVSGRTFSYLALGWFRQAPGKEREFVAAASWGGGSTGYADSVKGRFAISRDNVKNTQYLQMNSLKPEDTAVYYCVVGRRFKGSVYYTPNEYEYWGQGTQVTVSS

SEQ ID NO: 5 - protein, 126 aa, synthetic construct
QVQLVESGGGLVQAGGSLRLSCAVSGRTFSYLAMGWFRQAPGKEREFVAASSWGGGTSGYADSVKGRFAISRDNAKNTQYLQMNSLKPEDTAVYYCVVGRRFKGSVYYTPNEYEYWGQGTQVTVSS

SEQ ID NO: 6 - DNA, 378 bp, synthetic construct
  source 1..378: mol_type = other DNA
caggtgcagctggtggagagcggcggcggcctggtgcaggccggcggcagcctgaggctgagctgcgccgccagcggcggcaccttcaggatctacgccatgggctggttcaggcaggcccccggcaaggagagggagttcgtgggcagcatcagcatgatgaggggcatcaccgactacgccgagagcgtgaagggcaggttcaccatcagcagggacaacgccaagttcaccatgtacctgcagatgaacagcctgaagagcgaggacaccgccgtgtactactgcgccaaggccgtggacaagagcccctacggcggctggggctggggcccctacgacgactggggccagggcacccaggtgaccgtgagcagc

SEQ ID NO: 7 - DNA, 381 bp, synthetic construct
  source 1..381: mol_type = other DNA
caggtgcagctggtggagagcggcggcggcctggtgcaggccggcgacagcctgaggctgagctgcgccgccagcggcggcaccttcaggatctacgccatgggctggttcaggcaggcccccggcaaggagagggagttcgtgggcagcatcagcatgatgaggggcatcaccgactacgccgagagcgtgaagggcaggttcaccatcagcagggacaacgccaagttcaccatgtacctgcagatgaacaccctgaagcccgaggacaccgccgtgtactactgcgccatcagggagaggcccccccccatgggctggggcctggccggcatcagctacgactactggggccagggcacccaggtgaccgtgagcagc

SEQ ID NO: 8 - DNA, 381 bp, synthetic construct
  source 1..381: mol_type = other DNA
caggtgcagctggtggagagcggcggcggcctggtgcagcccggcggcagcctgaggctgagctgcgccgccagcggcaggaccttcaggatctacgccatgggctggttcaggcaggcccccggcaaggagagggagttcgtgggcagcatcaggctgatgaggggcatcaccgactacgccgacagcgtgaagggcaggttcaccatcagcagggacaacgccaagttcaccatgtacctgcagatgaacaccctgaagcccgaggacaccgccgtgtactactgcgccgccgtgggcagcggcggcgacttctacacccccagcaccagcggcgagtacaggtactggggccagggcacccaggtgaccgtgagcagc

SEQ ID NO: 9 - DNA, 378 bp, synthetic construct
  source 1..378: mol_type = other DNA
caggtgcagctggtggagagcggcggcggcctggtgcagcccggcggcagcctgaggctgagctgcgaggtgagcggcaggaccttcagctacctggccctgggctggttcaggcaggcccccggcaaggagagggagttcgtggccgccgccagctggggcggcggcagcaccggctacgccgacagcgtgaagggcaggttcgccatcagcagggacaacgtgaagaacacccagtacctgcagatgaacagcctgaagcccgaggacaccgccgtgtactactgcgtggtgggcaggaggttcaagggcagcgtgtactacacccccaacgagtacgagtactggggccagggcacccaggtgaccgtgagcagc

SEQ ID NO: 10 - DNA, 378 bp, synthetic construct
  source 1..378: mol_type = other DNA
caggtgcagctggtggagagcggcggcggcctggtgcaggccggcggcagcctgaggctgagctgcgccgtgagcggcaggaccttcagctacctggccatgggctggttcaggcaggcccccggcaaggagagggagttcgtggccgccagcagctggggcggcggcaccagcggctacgccgacagcgtgaagggcaggttcgccatcagcagggacaacgccaagaacacccagtacctgcagatgaacagcctgaagcccgaggacaccgccgtgtactactgcgtggtgggcaggaggttcaagggcagcgtgtactacacccccaacgagtacgagtactggggccagggcacccaggtgaccgtgagcagc

SEQ ID NO: 11 - protein, 8 aa, synthetic construct
GGTFRIYA

SEQ ID NO: 12 - protein, 8 aa, synthetic construct
GRTFSYLA

SEQ ID NO: 13 - protein, 8 aa, synthetic construct
GRTFRIYA

SEQ ID NO: 14 - protein, 8 aa, synthetic construct
ASWGGGST

SEQ ID NO: 15 - protein, 8 aa, synthetic construct
IRLMRGIT

SEQ ID NO: 16 - protein, 8 aa, synthetic construct
ISMMRGIT

SEQ ID NO: 17 - protein, 8 aa, synthetic construct
SSWGGGTS

SEQ ID NO: 18 - protein, 20 aa, synthetic construct
AAVGSGGDFYTPSTSGEYRY

SEQ ID NO: 19 - protein, 20 aa, synthetic construct
AIRERPPPMGWGLAGISYDY

SEQ ID NO: 20 - protein, 19 aa, synthetic construct
AKAVDKSPYGGWGWGPYDD

SEQ ID NO: 21 - protein, 19 aa, synthetic construct
VVGRRFKGSVYYTPNEYEY

SEQ ID NO: 22 - protein, 25 aa, synthetic construct
QVQLVESGGGLVQAGDSLRLSCAAS

SEQ ID NO: 23 - protein, 25 aa, synthetic construct
QVQLVESGGGLVQAGGSLRLSCAAS

SEQ ID NO: 24 - protein, 25 aa, synthetic construct
QVQLVESGGGLVQAGGSLRLSCAVS

SEQ ID NO: 25 - protein, 25 aa, synthetic construct
QVQLVESGGGLVQPGGSLRLSCAAS

SEQ ID NO: 26 - protein, 25 aa, synthetic construct
QVQLVESGGGLVQPGGSLRLSCEVS

SEQ ID NO: 27 - protein, 17 aa, synthetic construct
LGWFRQAPGKEREFVAA

SEQ ID NO: 28 - protein, 17 aa, synthetic construct
MGWFRQAPGKEREFVAA

SEQ ID NO: 29 - protein, 17 aa, synthetic construct
MGWFRQAPGKEREFVGS

SEQ ID NO: 30 - protein, 38 aa, synthetic construct
DYADSVKGRFTISRDNAKFTMYLQMNTLKPEDTAVYYC

SEQ ID NO: 31 - protein, 38 aa, synthetic construct
DYAESVKGRFTISRDNAKFTMYLQMNSLKSEDTAVYYC

SEQ ID NO: 32 - protein, 38 aa, synthetic construct
DYAESVKGRFTISRDNAKFTMYLQMNTLKPEDTAVYYC

SEQ ID NO: 33 - protein, 38 aa, synthetic construct
GYADSVKGRFAISRDNAKNTQYLQMNSLKPEDTAVYYC

SEQ ID NO: 34 - protein, 38 aa, synthetic construct
GYADSVKGRFAISRDNVKNTQYLQMNSLKPEDTAVYYC

SEQ ID NO: 35 - protein, 11 aa, synthetic construct
WGQGTQVTVSS

SEQ ID NO: 36 - protein, 25 aa, synthetic construct
QVQLVESGGGSVQAGGSLRLSCAAS

SEQ ID NO: 37 - protein, 8 aa, synthetic construct
DGTYRRYC

SEQ ID NO: 38 - protein, 17 aa, synthetic construct
MGWFRQAPGKEREKVAA

SEQ ID NO: 39 - protein, 8 aa, synthetic construct
IYTGDGTT

SEQ ID NO: 40 - protein, 38 aa, synthetic construct
YYADSVKGRFTISQENAKNTMYLQMNSLKPEDTAMYYC

SEQ ID NO: 41 - protein, 18 aa, synthetic construct
AADRSGCSVAWSYSSFED

SEQ ID NO: 42 - protein, 11 aa, synthetic construct
WGQGTQVTVSS

SEQ ID NO: 43 - protein, 125 aa, synthetic construct
QVQLVESGGGSVQAGGSLRLSCAASDGTYRRYCMGWFRQAPGKEREKVAAIYTGDGTTYYADSVKGRFTISQENAKNTMYLQMNSLKPEDTAMYYCAADRSGCSVAWSYSSFEDWGQGTQVTVSS

SEQ ID NO: 44 - DNA, 375 bp, synthetic construct
  source 1..375: mol_type = other DNA
caggtgcagctggtggagagcggcggcggcagcgtgcaggccggcggcagcctgaggctgagctgcgccgccagcgacggcacctacaggaggtactgcatgggctggttcaggcaggcccccggcaaggagagggagaaggtggccgccatctacaccggcgacggcaccacctactacgccgacagcgtgaagggcaggttcaccatcagccaggagaacgccaagaacaccatgtacctgcagatgaacagcctgaagcccgaggacaccgccatgtactactgcgccgccgacaggagcggctgcagcgtggcctggagctacagcagcttcgaggactggggccagggcacccaggtgaccgtgagcagc

SEQ ID NO: 45 - protein, 267 aa, synthetic construct
QVQLVESGGGLVKPGGSLRLSCAASDATYRRYCMGWFRQAPGKEREKVAAIYTGDATTYYADSVKGRFTISQENAKNTMYLQMNSLKPEDTAMYYCAADRSGCSVAFSYSSFEDWGQGTLVTVSSGGGGSGGGGSGGGGSQVQLVESGGGLVQAGGSLRLSCAASGRTFSSYAMGWFRQAPGKEREFVAGISWSGDSTYYADSVKGRFTISRDNAKNTVGLQMNSLKPEDTAVYYCAAASGQVQTVVVVTDRFYHYWGQGTQVTVSS

SEQ ID NO: 46 - DNA, 801 bp, synthetic construct
  source 1..801: mol_type = other DNA
caggtgcagctggtggagagcggcggcggcctggtgaagcccggcggcagcctgaggctgagctgcgccgccagcgacgccacctacaggaggtactgcatgggctggttcaggcaggcccccggcaaggagagggagaaggtggccgccatctacaccggcgacgccaccacctactacgccgacagcgtgaagggcaggttcaccatcagccaggagaacgccaagaacaccatgtacctgcagatgaacagcctgaagcccgaggacaccgccatgtactactgcgccgccgacaggagcggctgcagcgtggccttcagctacagcagcttcgaggactggggccagggcaccctggtgaccgtgagcagcggcggcggcggcagcggcggcggcggcagcggcggcggcggcagccaggtgcagctggtggagagcggcggcggcctggtgcaggccggcggcagcctgaggctgagctgcgccgccagcggcaggaccttcagcagctacgccatgggctggttcaggcaggcccccggcaaggagagggagttcgtggccggcatcagctggagcggcgacagcacctactacgccgacagcgtgaagggcaggttcaccatcagcagggacaacgccaagaacaccgtgggcctgcagatgaacagcctgaagcccgaggacaccgccgtgtactactgcgccgccgccagcggccaggtgcagaccgtggtggtggtgaccgacaggttctaccactactggggccagggcacccaggtgaccgtgagcagc

SEQ ID NO: 47 - protein, 408 aa, synthetic construct
QVQLVESGGGLVKPGGSLRLSCAASDATYRRYCMGWFRQAPGKEREKVAAIYTGDATTYYADSVKGRFTISQENAKNTMYLQMNSLKPEDTAMYYCAADRSGCSVAFSYSSFEDWGQGTLVTVSSGGGGSGGGGSGGGGSQVQLVESGGGLVQAGGSLRLSCAASGRTFSSYAMGWFRQAPGKEREFVAGISWSGDSTYYADSVKGRFTISRDNAKNTVGLQMNSLKPEDTAVYYCAAASGQVQTVVVVTDRFYHYWGQGTQVTVSSGGGGSGGGGSGGGGSQVQLVESGGGLVQAGGSLRLSCAASGGTFRIYAMGWFRQAPGKEREFVGSISMMRGITDYAESVKGRFTISRDNAKFTMYLQMNSLKSEDTAVYYCAKAVDKSPYGGWGWGPYDDWGQGTQVTVSS

SEQ ID NO: 48 - protein, 409 aa, synthetic construct
QVQLVESGGGLVKPGGSLRLSCAASDATYRRYCMGWFRQAPGKEREKVAAIYTGDATTYYADSVKGRFTISQENAKNTMYLQMNSLKPEDTAMYYCAADRSGCSVAFSYSSFEDWGQGTLVTVSSGGGGSGGGGSGGGGSQVQLVESGGGLVQAGGSLRLSCAASGRTFSSYAMGWFRQAPGKEREFVAGISWSGDSTYYADSVKGRFTISRDNAKNTVGLQMNSLKPEDTAVYYCAAASGQVQTVVVVTDRFYHYWGQGTQVTVSSGGGGSGGGGSGGGGSQVQLVESGGGLVQAGDSLRLSCAASGGTFRIYAMGWFRQAPGKEREFVGSISMMRGITDYAESVKGRFTISRDNAKFTMYLQMNTLKPEDTAVYYCAIRERPPPMGWGLAGISYDYWGQGTQVTVSS

SEQ ID NO: 49 - protein, 409 aa, synthetic construct
QVQLVESGGGLVKPGGSLRLSCAASDATYRRYCMGWFRQAPGKEREKVAAIYTGDATTYYADSVKGRFTISQENAKNTMYLQMNSLKPEDTAMYYCAADRSGCSVAFSYSSFEDWGQGTLVTVSSGGGGSGGGGSGGGGSQVQLVESGGGLVQAGGSLRLSCAASGRTFSSYAMGWFRQAPGKEREFVAGISWSGDSTYYADSVKGRFTISRDNAKNTVGLQMNSLKPEDTAVYYCAAASGQVQTVVVVTDRFYHYWGQGTQVTVSSGGGGSGGGGSGGGGSQVQLVESGGGLVQPGGSLRLSCAASGRTFRIYAMGWFRQAPGKEREFVGSIRLMRGITDYADSVKGRFTISRDNAKFTMYLQMNTLKPEDTAVYYCAAVGSGGDFYTPSTSGEYRYWGQGTQVTVSS

SEQ ID NO: 50 - protein, 408 aa, synthetic construct
QVQLVESGGGLVKPGGSLRLSCAASDATYRRYCMGWFRQAPGKEREKVAAIYTGDATTYYADSVKGRFTISQENAKNTMYLQMNSLKPEDTAMYYCAADRSGCSVAFSYSSFEDWGQGTLVTVSSGGGGSGGGGSGGGGSQVQLVESGGGLVQAGGSLRLSCAASGRTFSSYAMGWFRQAPGKEREFVAGISWSGDSTYYADSVKGRFTISRDNAKNTVGLQMNSLKPEDTAVYYCAAASGQVQTVVVVTDRFYHYWGQGTQVTVSSGGGGSGGGGSGGGGSQVQLVESGGGLVQPGGSLRLSCEVSGRTFSYLALGWFRQAPGKEREFVAAASWGGGSTGYADSVKGRFAISRDNVKNTQYLQMNSLKPEDTAVYYCVVGRRFKGSVYYTPNEYEYWGQGTQVTVSS

SEQ ID NO: 51 - protein, 408 aa, synthetic construct
QVQLVESGGGLVKPGGSLRLSCAASDATYRRYCMGWFRQAPGKEREKVAAIYTGDATTYYADSVKGRFTISQENAKNTMYLQMNSLKPEDTAMYYCAADRSGCSVAFSYSSFEDWGQGTLVTVSSGGGGSGGGGSGGGGSQVQLVESGGGLVQAGGSLRLSCAASGRTFSSYAMGWFRQAPGKEREFVAGISWSGDSTYYADSVKGRFTISRDNAKNTVGLQMNSLKPEDTAVYYCAAASGQVQTVVVVTDRFYHYWGQGTQVTVSSGGGGSGGGGSGGGGSQVQLVESGGGLVQAGGSLRLSCAVSGRTFSYLAMGWFRQAPGKEREFVAASSWGGGTSGYADSVKGRFAISRDNAKNTQYLQMNSLKPEDTAVYYCVVGRRFKGSVYYTPNEYEYWGQGTQVTVSS

SEQ ID NO: 52 - DNA, 1224 bp, synthetic construct
  source 1..1224: mol_type = other DNA
caggtgcagctggtggagagcggcggcggcctggtgaagcccggcggcagcctgaggctgagctgcgccgccagcgacgccacctacaggaggtactgcatgggctggttcaggcaggcccccggcaaggagagggagaaggtggccgccatctacaccggcgacgccaccacctactacgccgacagcgtgaagggcaggttcaccatcagccaggagaacgccaagaacaccatgtacctgcagatgaacagcctgaagcccgaggacaccgccatgtactactgcgccgccgacaggagcggctgcagcgtggccttcagctacagcagcttcgaggactggggccagggcaccctggtgaccgtgagcagcggcggcggcggcagcggcggcggcggcagcggcggcggcggcagccaggtgcagctggtggagagcggcggcggcctggtgcaggccggcggcagcctgaggctgagctgcgccgccagcggcaggaccttcagcagctacgccatgggctggttcaggcaggcccccggcaaggagagggagttcgtggccggcatcagctggagcggcgacagcacctactacgccgacagcgtgaagggcaggttcaccatcagcagggacaacgccaagaacaccgtgggcctgcagatgaacagcctgaagcccgaggacaccgccgtgtactactgcgccgccgccagcggccaggtgcagaccgtggtggtggtgaccgacaggttctaccactactggggccagggcacccaggtgaccgtgagcagcggcggcggcggcagcggcggcggcggcagcggcggcggcggcagccaggtgcagctggtggagagcggcggcggcctggtgcaggccggcggcagcctgaggctgagctgcgccgccagcggcggcaccttcaggatctacgccatgggctggttcaggcaggcccccggcaaggagagggagttcgtgggcagcatcagcatgatgaggggcatcaccgactacgccgagagcgtgaagggcaggttcaccatcagcagggacaacgccaagttcaccatgtacctgcagatgaacagcctgaagagcgaggacaccgccgtgtactactgcgccaaggccgtggacaagagcccctacggcggctggggctggggcccctacgacgactggggccagggcacccaggtgaccgtgagcagc

SEQ ID NO: 53 - DNA, 1227 bp, synthetic construct
  source 1..1227: mol_type = other DNA
caggtgcagctggtggagagcggcggcggcctggtgaagcccggcggcagcctgaggctgagctgcgccgccagcgacgccacctacaggaggtactgcatgggctggttcaggcaggcccccggcaaggagagggagaaggtggccgccatctacaccggcgacgccaccacctactacgccgacagcgtgaagggcaggttcaccatcagccaggagaacgccaagaacaccatgtacctgcagatgaacagcctgaagcccgaggacaccgccatgtactactgcgccgccgacaggagcggctgcagcgtggccttcagctacagcagcttcgaggactggggccagggcaccctggtgaccgtgagcagcggcggcggcggcagcggcggcggcggcagcggcggcggcggcagccaggtgcagctggtggagagcggcggcggcctggtgcaggccggcggcagcctgaggctgagctgcgccgccagcggcaggaccttcagcagctacgccatgggctggttcaggcaggcccccggcaaggagagggagttcgtggccggcatcagctggagcggcgacagcacctactacgccgacagcgtgaagggcaggttcaccatcagcagggacaacgccaagaacaccgtgggcctgcagatgaacagcctgaagcccgaggacaccgccgtgtactactgcgccgccgccagcggccaggtgcagaccgtggtggtggtgaccgacaggttctaccactactggggccagggcacccaggtgaccgtgagcagcggcggcggcggcagcggcggcggcggcagcggcggcggcggcagccaggtgcagctggtggagagcggcggcggcctggtgcaggccggcgacagcctgaggctgagctgcgccgccagcggcggcaccttcaggatctacgccatgggctggttcaggcaggcccccggcaaggagagggagttcgtgggcagcatcagcatgatgaggggcatcaccgactacgccgagagcgtgaagggcaggttcaccatcagcagggacaacgccaagttcaccatgtacctgcagatgaacaccctgaagcccgaggacaccgccgtgtactactgcgccatcagggagaggcccccccccatgggctggggcctggccggcatcagctacgactactggggccagggcacccaggtgaccgtgagcagc

SEQ ID NO: 54 - DNA, 1227 bp, synthetic construct
  source 1..1227: mol_type = other DNA
caggtgcagctggtggagagcggcggcggcctggtgaagcccggcggcagcctgaggctgagctgcgccgccagcgacgccacctacaggaggtactgcatgggctggttcaggcaggcccccggcaaggagagggagaaggtggccgccatctacaccggcgacgccaccacctactacgccgacagcgtgaagggcaggttcaccatcagccaggagaacgccaagaacaccatgtacctgcagatgaacagcctgaagcccgaggacaccgccatgtactactgcgccgccgacaggagcggctgcagcgtggccttcagctacagcagcttcgaggactggggccagggcaccctggtgaccgtgagcagcggcggcggcggcagcggcggcggcggcagcggcggcggcggcagccaggtgcagctggtggagagcggcggcggcctggtgcaggccggcggcagcctgaggctgagctgcgccgccagcggcaggaccttcagcagctacgccatgggctggttcaggcaggcccccggcaaggagagggagttcgtggccggcatcagctggagcggcgacagcacctactacgccgacagcgtgaagggcaggttcaccatcagcagggacaacgccaagaacaccgtgggcctgcagatgaacagcctgaagcccgaggacaccgccgtgtactactgcgccgccgccagcggccaggtgcagaccgtggtggtggtgaccgacaggttctaccactactggggccagggcacccaggtgaccgtgagcagcggcggcggcggcagcggcggcggcggcagcggcggcggcggcagccaggtgcagctggtggagagcggcggcggcctggtgcagcccggcggcagcctgaggctgagctgcgccgccagcggcaggaccttcaggatctacgccatgggctggttcaggcaggcccccggcaaggagagggagttcgtgggcagcatcaggctgatgaggggcatcaccgactacgccgacagcgtgaagggcaggttcaccatcagcagggacaacgccaagttcaccatgtacctgcagatgaacaccctgaagcccgaggacaccgccgtgtactactgcgccgccgtgggcagcggcggcgacttctacacccccagcaccagcggcgagtacaggtactggggccagggcacccaggtgaccgtgagcagc

SEQ ID NO: 55 - DNA, 1224 bp, synthetic construct
  source 1..1224: mol_type = other DNA
caggtgcagctggtggagagcggcggcggcctggtgaagcccggcggcagcctgaggctgagctgcgccgccagcgacgccacctacaggaggtactgcatgggctggttcaggcaggcccccggcaaggagagggagaaggtggccgccatctacaccggcgacgccaccacctactacgccgacagcgtgaagggcaggttcaccatcagccaggagaacgccaagaacaccatgtacctgcagatgaacagcctgaagcccgaggacaccgccatgtactactgcgccgccgacaggagcggctgcagcgtggccttcagctacagcagcttcgaggactggggccagggcaccctggtgaccgtgagcagcggcggcggcggcagcggcggcggcggcagcggcggcggcggcagccaggtgcagctggtggagagcggcggcggcctggtgcaggccggcggcagcctgaggctgagctgcgccgccagcggcaggaccttcagcagctacgccatgggctggttcaggcaggcccccggcaaggagagggagttcgtggccggcatcagctggagcggcgacagcacctactacgccgacagcgtgaagggcaggttcaccatcagcagggacaacgccaagaacaccgtgggcctgcagatgaacagcctgaagcccgaggacaccgccgtgtactactgcgccgccgccagcggccaggtgcagaccgtggtggtggtgaccgacaggttctaccactactggggccagggcacccaggtgaccgtgagcagcggcggcggcggcagcggcggcggcggcagcggcggcggcggcagccaggtgcagctggtggagagcggcggcggcctggtgcagcccggcggcagcctgaggctgagctgcgaggtgagcggcaggaccttcagctacctggccctgggctggttcaggcaggcccccggcaaggagagggagttcgtggccgccgccagctggggcggcggcagcaccggctacgccgacagcgtgaagggcaggttcgccatcagcagggacaacgtgaagaacacccagtacctgcagatgaacagcctgaagcccgaggacaccgccgtgtactactgcgtggtgggcaggaggttcaagggcagcgtgtactacacccccaacgagtacgagtactggggccagggcacccaggtgaccgtgagcagc

SEQ ID NO: 56 - DNA, 1224 bp, synthetic construct
  source 1..1224: mol_type = other DNA
caggtgcagctggtggagagcggcggcggcctggtgaagcccggcggcagcctgaggctgagctgcgccgccagcgacgccacctacaggaggtactgcatgggctggttcaggcaggcccccggcaaggagagggagaaggtggccgccatctacaccggcgacgccaccacctactacgccgacagcgtgaagggcaggttcaccatcagccaggagaacgccaagaacaccatgtacctgcagatgaacagcctgaagcccgaggacaccgccatgtactactgcgccgccgacaggagcggctgcagcgtggccttcagctacagcagcttcgaggactggggccagggcaccctggtgaccgtgagcagcggcggcggcggcagcggcggcggcggcagcggcggcggcggcagccaggtgcagctggtggagagcggcggcggcctggtgcaggccggcggcagcctgaggctgagctgcgccgccagcggcaggaccttcagcagctacgccatgggctggttcaggcaggcccccggcaaggagagggagttcgtggccggcatcagctggagcggcgacagcacctactacgccgacagcgtgaagggcaggttcaccatcagcagggacaacgccaagaacaccgtgggcctgcagatgaacagcctgaagcccgaggacaccgccgtgtactactgcgccgccgccagcggccaggtgcagaccgtggtggtggtgaccgacaggttctaccactactggggccagggcacccaggtgaccgtgagcagcggcggcggcggcagcggcggcggcggcagcggcggcggcggcagccaggtgcagctggtggagagcggcggcggcctggtgcaggccggcggcagcctgaggctgagctgcgccgtgagcggcaggaccttcagctacctggccatgggctggttcaggcaggcccccggcaaggagagggagttcgtggccgccagcagctggggcggcggcaccagcggctacgccgacagcgtgaagggcaggttcgccatcagcagggacaacgccaagaacacccagtacctgcagatgaacagcctgaagcccgaggacaccgccgtgtactactgcgtggtgggcaggaggttcaagggcagcgtgtactacacccccaacgagtacgagtactggggccagggcacccaggtgaccgtgagcagc

SEQ ID NO: 57 - protein, 25 aa, synthetic construct
QVQLVESGGGLVKPGGSLRLSCAAS

SEQ ID NO: 58 - protein, 8 aa, synthetic construct
DATYRRYC

SEQ ID NO: 59 - protein, 8 aa, synthetic construct
IYTGDATT

SEQ ID NO: 60 - protein, 18 aa, synthetic construct
AADRSGCSVAFSYSSFED

SEQ ID NO: 61 - protein, 11 aa, synthetic construct
WGQGTLVTVSS

SEQ ID NO: 62 - protein, 25 aa, synthetic construct
QVQLVESGGGLVQAGGSLRLSCAAS

SEQ ID NO: 63 - protein, 8 aa, synthetic construct
GRTFSSYA

SEQ ID NO: 64 - protein, 17 aa, synthetic construct
MGWFRQAPGKEREFVAG

SEQ ID NO: 65 - protein, 8 aa, synthetic construct
ISWSGDST

SEQ ID NO: 66 - protein, 38 aa, synthetic construct
YYADSVKGRFTISRDNAKNTVGLQMNSLKPEDTAVYYC

SEQ ID NO: 67 - protein, 20 aa, synthetic construct
AAASGQVQTVVVVTDRWYHY

SEQ ID NO: 68 - protein, 11 aa, synthetic construct
WGQGTQVTVSS

SEQ ID NO: 69 - protein, 127 aa, synthetic construct
QVQLVESGGGLVQAGGSLRLSCAASGRTFSSYAMGWFRQAPGKEREFVAGISWSGDSTYYADSVKGRFTISRDNAKNTVGLQMNSLKPEDTAVYYCAAASGQVQTVVVVTDRWYHYWGQGTQVTVSS

SEQ ID NO: 70 - protein, 20 aa, synthetic construct
AAASGQVQTVVVVTDRFYHY